European Patent Specification EP 3 434 101 B1, published August 16, 2023. Title: NON-HUMAN ANIMALS HAVING A HUMANIZED SIGNAL-REGULATORY PROTEIN GENE. Applicant: Regeneron Pharmaceuticals, Inc. Application tba. The sequence listing filed with the application follows.

SEQUENCE LISTING (8 sequences)

SEQ ID NO: 1 - DNA, 4007 bp, Mus musculus
gcgctcggccgggccgccctcgcgctggcctcgcgacggctccgcacagcccgcactcgctctgcgagctgtccccgctcgcgcttgctctccgatctccgtccccgctccctctccctcttcctctccccctctttccttctccctcgctatccgctcccccgcccccgtgcctctggctctgcgcctggctccctcgggtccgctcccctttcccgccggcctggcccggcgtcacgctcccggagtctccccgctcggcggcgtctcattgtgggagggggtcagatcaccccgccgggcggtggcgctggggggcagcggagggggaggggccttagtcgttcgcccgcgccgcccgcccgcctgccgagcgcgctcaccgccgctctccctccttgctctgcagccgcggcccatggagcccgccggcccggcccctggccgcctagggccgctgctgctctgcctgctgctctccgcgtcctgtttctgtacaggagccacggggaaggaactgaaggtgactcagcctgagaaatcagtgtctgttgctgctggggattcgaccgttctgaactgcactttgacctccttgttgccggtgggacccattaggtggtacagaggagtagggccaagccggctgttgatctacagtttcgcaggagaatacgttcctcgaattagaaatgtttcagatactactaagagaaacaatatggacttttccatccgtatcagtaatgtcaccccagcagatgctggcatctactactgtgtgaagttccagaaaggatcatcagagcctgacacagaaatacaatctggagggggaacagaggtctatgtactcgccaaaccttctccaccggaggtatccggcccagcagacaggggcatacctgaccagaaagtgaacttcacctgcaagtctcatggcttctctccccggaatatcaccctgaagtggttcaaagatgggcaagaactccaccccttggagaccaccgtgaaccctagtggaaagaatgtctcctacaacatctccagcacagtcagggtggtactaaactccatggatgttaattctaaggtcatctgcgaggtagcccacatcaccttggatagaagccctcttcgtgggattgctaacctgtctaacttcatccgagtttcacccaccgtgaaggtcacccaacagtccccgacgtcaatgaaccaggtgaacctcacctgccgggctgagaggttctaccccgaggatctccagctgatctggctggagaatggaaacgtatcacggaatgacacgcccaagaatctcacaaagaacacggatgggacctataattacacaagcttgttcctggtgaactcatctgctcatagagaggacgtggtgttcacgtgccaggtgaagcacgaccaacagccagcgatcacccgaaaccataccgtgctgggatttgcccactcgagtgatcaagggagcatgcaaaccttccctgataataatgctacccacaactggaatgtcttcatcggtgtgggcgtggcgtgtgctttgctcgtagtcctgctgatggctgctctctacctcctccggatcaaacagaagaaagccaaggggtcaacatcttccacacggttgcacgagcccgagaagaacgccagggaaataacccagatccaggacacaaatgacatcaacgacatcacatacgcagacctgaatctgcccaaagagaagaagcccgcaccccgggcccctgagcctaacaaccacacagaatatgcaagcattgagacaggcaaagtgcctaggccagaggataccctcacctatgctgacctggacatggtccacctcagccgggcacagccagcccccaagcctgagccatctttctcagagtatgctagtgtccaggtccagaggaagtgaatggggctgtggtctgtactaggccccatccccacaagttttcttgtcctacatggagtggccatgacgaggacatccagccagccaatcctgtccccagaaggccaggtggcacgggtcctaggaccaggggtaagggtggcctttgtcttccctccgtggctcttcaacacctcttgggcacccacgtccccttcttccggaggctgggtgttgcagaaccagagggcgaactggagaaagctgcctggaatccaagaagtgttgtgcctcggcccatcactcgtgggtctggatcctggtcttggcaaccccaggttgcgtccttgatgttccagagcttggtcttctgtgtggagaagagctcaccatctctacccaacttgagctttgggaccagactccctttagatcaaaccgccccatctgtggaagaactacaccagaagtcagcaagttttcagccaacagtgctggcctccccacctcccaggctgactagccctggggagaaggaaccctctcctcctagaccagcagagactccctgggcatgttcagtgtggccccacctcccttccagtcccagcttgcttcctccagctagcactaactcagcagcatcgctctgtggacgcctgtaaattattgagaaatgtgaactgtgcagtcttaaagctaaggtgttagaaaatttgatttatgctgtttagttgttgttgggtttcttttctttttaatttctttttcttttttgattttttttctttcccttaaaacaacagcagcagcatcttggctctttgtcatgtgttgaatggttgggtcttgtgaagtctgaggtctaacagtttattgtcctggaaggattttcttacagcagaaacagatttttttcaaattcccagaatcctgaggaccaagaaggatccctcagctgctacttccagcacccagcgtcactgggacgaaccaggccctgttcttacaaggccacatggctggccctttgcctccatggctactgtggtaagtgcagccttgtctgacccaatgctgacctaatgttggccattccacattgaggggacaaggtcagtgatgccccccttcactcacaagcacttcagaggcatgcagagagaagggacactcggccagctctctgaggtaatcagtgcaaggaggagtccgttttttgccagcaaacctcagcaggatcacactggaacagaacctggtcatacctgtgacaacacagctgtgagccagggcaaaccacccactgtcactggctcgagagtctgggcagaggctctgaccctccaccctttaaactggatgccggggcctggctgggcccaatgccaagtggttatggcaaccctgactatctggtcttaacatgtagctcaggaagtggaggcgctaatgtccccaatccctggggattcctgattccagctattcatgtaagcagagccaacctgcctatttctgtaggtgcgactgggatgttaggagcacagcaaggacccagctctgtagggctggtgacctgatacttctcataatggcatctagaagttaggctgagttggcctcactggcccagcaaaccagaacttgtctttgtccgggccatgttcttgggctgtcttctaattccaaagggttggttggtaaagctccacccccttctcctctgcctaaagacatcacatgtgtatacacacacgggtgtatagatgagttaaaagaatgtcctcgctggcatcctaattttgtcttaagtttttttggagggagaaaggaacaaggcaagggaagatgtgtagctttggctttaaccaggcagcctgggggctcccaagcctatggaaccctggtacaaagaagagaacagaagcgccctgtgaggagtgggatttgtttttctgtagaccagatgagaaggaaacaggccctgttttgtacatagttgcaacttaaaatttttggcttgcaaaatatttttgtaataaagatttctgggtaacaataaaaaaaaaaaaaaaaa

SEQ ID NO: 2 - protein, 509 aa, Mus musculus
MEPAGPAPGRLGPLLLCLLLSASCFCTGATGKELKVTQPEKSVSVAAGDSTVLNCTLTSLLPVGPIRWYRGVGPSRLLIYSFAGEYVPRIRNVSDTTKRNNMDFSIRISNVTPADAGIYYCVKFQKGSSEPDTEIQSGGGTEVYVLAKPSPPEVSGPADRGIPDQKVNFTCKSHGFSPRNITLKWFKDGQELHPLETTVNPSGKNVSYNISSTVRVVLNSMDVNSKVICEVAHITLDRSPLRGIANLSNFIRVSPTVKVTQQSPTSMNQVNLTCRAERFYPEDLQLIWLENGNVSRNDTPKNLTKNTDGTYNYTSLFLVNSSAHREDVVFTCQVKHDQQPAITRNHTVLGFAHSSDQGSMQTFPDNNATHNWNVFIGVGVACALLVVLLMAALYLLRIKQKKAKGSTSSTRLHEPEKNAREITQIQDTNDINDITYADLNLPKEKKPAPRAPEPNNHTEYASIETGKVPRPEDTLTYADLDMVHLSRAQPAPKPEPSFSEYASVQVQRK

SEQ ID NO: 3 - DNA, 4201 bp, Homo sapiens
tccggcccgcacccacccccaagaggggccttcagctttggggctcagaggcacgacctcctggggagggttaaaaggcagacgcccccccgccccccgcgcccccgcgccccgactccttcgccgcctccagcctctcgccagtgggaagcggggagcagccgcgcggccggagtccggaggcgaggggaggtcggccgcaacttccccggtccaccttaagaggacgatgtagccagctcgcagcgctgaccttagaaaaacaagtttgcgcaaagtggagcggggacccggcctctgggcagccccggcggcgcttccagtgccttccagccctcgcgggcggcgcagccgcggcccatggagcccgccggcccggcccccggccgcctcgggccgctgctctgcctgctgctcgccgcgtcctgcgcctggtcaggagtggcgggtgaggaggagctgcaggtgattcagcctgacaagtccgtgttggttgcagctggagagacagccactctgcgctgcactgcgacctctctgatccctgtggggcccatccagtggttcagaggagctggaccaggccgggaattaatctacaatcaaaaagaaggccacttcccccgggtaacaactgtttcagacctcacaaagagaaacaacatggacttttccatccgcatcggtaacatcaccccagcagatgccggcacctactactgtgtgaagttccggaaagggagccccgatgacgtggagtttaagtctggagcaggcactgagctgtctgtgcgcgccaaaccctctgcccccgtggtatcgggccctgcggcgagggccacacctcagcacacagtgagcttcacctgcgagtcccacggcttctcacccagagacatcaccctgaaatggttcaaaaatgggaatgagctctcagacttccagaccaacgtggaccccgtaggagagagcgtgtcctacagcatccacagcacagccaaggtggtgctgacccgcgaggacgttcactctcaagtcatctgcgaggtggcccacgtcaccttgcagggggaccctcttcgtgggactgccaacttgtctgagaccatccgagttccacccaccttggaggttactcaacagcccgtgagggcagagaaccaggtgaatgtcacctgccaggtgaggaagttctacccccagagactacagctgacctggttggagaatggaaacgtgtcccggacagaaacggcctcaaccgttacagagaacaaggatggtacctacaactggatgagctggctcctggtgaatgtatctgcccacagggatgatgtgaagctcacctgccaggtggagcatgacgggcagccagcggtcagcaaaagccatgacctgaaggtctcagcccacccgaaggagcagggctcaaataccgccgctgagaacactggatctaatgaacggaacatctatattgtggtgggtgtggtgtgcaccttgctggtggccctactgatggcggccctctacctcgtccgaatcagacagaagaaagcccagggctccacttcttctacaaggttgcatgagcccgagaagaatgccagagaaataacacaggacacaaatgatatcacatatgcagacctgaacctgcccaaggggaagaagcctgctccccaggctgcggagcccaacaaccacacggagtatgccagcattcagaccagcccgcagcccgcgtcggaggacaccctcacctatgctgacctggacatggtccacctcaaccggacccccaagcagccggcccccaagcctgagccgtccttctcagagtacgccagcgtccaggtcccgaggaagtgaatgggaccgtggtttgctctagcacccatctctacgcgctttcttgtcccacagggagccgccgtgatgagcacagccaacccagttcccggagggctggggcggtgcaggctctgggacccaggggccagggtggctcttctctccccacccctccttggctctccagcacttcctgggcagccacggccccctccccccacattgccacatacctggaggctgacgttgccaaaccagccagggaaccaacctgggaagtggccagaactgcctggggtccaagaactcttgtgcctccgtccatcaccatgtgggttttgaagaccctcgactgcctccccgatgctccgaagcctgatcttccagggtggggaggagaaaatcccacctcccctgacctccaccacctccaccaccaccaccaccaccaccaccaccactaccaccaccacccaactggggctagagtggggaagatttcccctttagatcaaactgccccttccatggaaaagctggaaaaaaactctggaacccatatccaggcttggtgaggttgctgccaacagtcctggcctcccccatccctaggctaaagagccatgagtcctggaggaggagaggacccctcccaaaggactggagacaaaaccctctgcttccttgggtccctccaagactccctggggcccaactgtgttgctccacccggacccatctctcccttctagacctgagcttgcccctccagctagcactaagcaacatctcgctgtggacgcctgtaaattactgagaaatgtgaaacgtgcaatcttgaaactgaggtgttagaaaacttgatctgtggtgttttgttttgttttttttcttaaaacaacagcaacgtgatcttggctgtctgtcatgtgttgaagtccatggttgggtcttgtgaagtctgaggtttaacagtttgttgtcctggagggattttcttacagcgaagacttgagttcctccaagtcccagaaccccaagaatgggcaagaaggatcaggtcagccactccctggagacacagccttctggctgggactgacttggccatgttctcagctgagccacgcggctggtagtgcagccttctgtgaccccgctgtggtaagtccagcctgcccagggctgctgagggctgcctcttgacagtgcagtcttatcgagacccaatgcctcagtctgctcatccgtaaagtggggatagtgaagatgacacccctccccaccacctctcataagcactttaggaacacacagagggtagggatagtggccctggccgtctatcctacccctttagtgaccgcccccatcccggctttctgagctgatccttgaagaagaaatcttccatttctgctctcaaaccctactgggatcaaactggaataaattgaagacagccagggggatggtgcagctgtgaagctcgggctgattccccctctgtcccagaaggttggccagagggtgtgacccagttaccctttaacccccacccttccagtcgggtgtgagggcctgaccgggcccagggcaagcagatgtcgcaagccctatttattcagtcttcactataactcttagagttgagacgctaatgttcatgactcctggccttgggatgcccaagggatttctggctcaggctgtaaaagtagctgagccatcctgcccattcctggaggtcctacaggtgaaactgcaggagctcagcatagacccagctctctgggggatggtcacctggtgatttcaatgatggcatccaggaattagctgagccaacagaccatgtggacagctttggccagagctcccgtgtggcatctgggagccacagtgacccagccacctggctcaggctagttccaaattccaaaagattggcttgtaaaccttcgtctccctctcttttacccagagacagcacatacgtgtgcacacgcatgcacacacacattcagtattttaaaagaatgttttcttggtgccattttcattttattttattttttaattcttggagggggaaataagggaataaggccaaggaagatgtatagctttagctttagcctggcaacctggagaatccacataccttgtgtattgaaccccaggaaaaggaagaggtcgaaccaaccctgcggaaggagcatggtttcaggagtttattttaagactgctgggaaggaaacaggccccattttgtatatagttgcaacttaaactttttggcttgcaaaatatttttgtaataaagatttctgggtaataatga

SEQ ID NO: 4 - protein, 504 aa, Homo sapiens
MEPAGPAPGRLGPLLCLLLAASCAWSGVAGEEELQVIQPDKSVLVAAGETATLRCTATSLIPVGPIQWFRGAGPGRELIYNQKEGHFPRVTTVSDLTKRNNMDFSIRIGNITPADAGTYYCVKFRKGSPDDVEFKSGAGTELSVRAKPSAPVVSGPAARATPQHTVSFTCESHGFSPRDITLKWFKNGNELSDFQTNVDPVGESVSYSIHSTAKVVLTREDVHSQVICEVAHVTLQGDPLRGTANLSETIRVPPTLEVTQQPVRAENQVNVTCQVRKFYPQRLQLTWLENGNVSRTETASTVTENKDGTYNWMSWLLVNVSAHRDDVKLTCQVEHDGQPAVSKSHDLKVSAHPKEQGSNTAAENTGSNERNIYIVVGVVCTLLVALLMAALYLVRIRQKKAQGSTSSTRLHEPEKNAREITQDTNDITYADLNLPKGKKPAPQAAEPNNHTEYASIQTSPQPASEDTLTYADLDMVHLNRTPKQPAPKPEPSFSEYASVQVPRK

SEQ ID NO: 5 - protein, 508 aa, Homo sapiens
MEPAGPAPGRLGPLLLCLLLSASCFCTGVAGEEELQVIQPDKSVLVAAGETATLRCTATSLIPVGPIQWFRGAGPGRELIYNQKEGHFPRVTTVSDLTKRNNMDFSIRIGNITPADAGTYYCVKFRKGSPDDVEFKSGAGTELSVRAKPSAPVVSGPAARATPQHTVSFTCESHGFSPRDITLKWFKNGNELSDFQTNVDPVGESVSYSIHSTAKVVLTREDVHSQVICEVAHVTLQGDPLRGTANLSETIRVPPTLEVTQQPVRAENQVNVTCQVRKFYPQRLQLTWLENGNVSRTETASTVTENKDGTYNWMSWLLVNVSAHRDDVKLTCQVEHDGQPAVSKSHDLKVSAHPKEQGSNTAADNNATHNWNVFIGVGVACALLVVLLMAALYLLRIKQKKAKGSTSSTRLHEPEKNAREITQIQDTNDINDITYADLNLPKEKKPAPRAPEPNNHTEYASIETGKVPRPEDTLTYADLDMVHLSRAQPAPKPEPSFSEYASVQVQRK

SEQ ID NO: 6 - DNA, 200 bp, Artificial Sequence
  Synthetic Oligonucleotide
agctctcctaccactagactgctgagacccgctgctctgctcaggactcgatttccagtacacaatctccctctttgaaaagtaccacacatcctggggtgctcttgcatttgtgtgacactttgctagccaggctcagtcctgggttccaggtggggactcaaacacactggcacgagtctacattggatattcttggt

SEQ ID NO: 7 - DNA, 199 bp, Artificial Sequence
  Synthetic Oligonucleotide
gctccccattcctcactggcccagcccctcttccctactctttctagcccctgcctcatctccctggctgccattgggagcctgccccactggaagccagtcgagataacttcgtataatgtatgctatacgaagttatatgcatggcctccgcgccgggttttggcgcctcccgcgggcgcccccctcctcacggcga

SEQ ID NO: 8 - DNA, 200 bp, Artificial Sequence
  Synthetic Oligonucleotide
cattctcagtattgttttgccaagttctaattccatcagacctcgacctgcagcccctagataacttcgtataatgtatgctatacgaagttatgctagctgtctcatagaggctggcgatctggctcagggacagccagtactgcaaagagtatccttgttcataccttctcctagtggccatctccctgggacagtca